European Patent Specification EP 2 734 552 B1, published November 13, 2024. Title: Antibodies. Applicant: CSL. The sequence listing filed with the application follows.

SEQUENCE LISTING (77 sequences)

SEQ ID NO: 1 - protein, 615 aa, Homo sapiens
MRALLLLGFLLVSLESTLSIPPWEAPKEHKYKAEEHTVVLTVTGEPCHFPFQYHRQLYHKCTHKGRPGPQPWCATTPNFDQDQRWGYCLEPKKVKDHCSKHSPCQKGGTCVNMPSGPHCLCPQHLTGNHCQKEKCFEPQLLRFFHKNEIWYRTEQAAVARCQCKGPDAHCQRLASQACRTNPCLHGGRCLEVEGHRLCHCPVGYTGAFCDVDTKASCYDGRGLSYRGLARTTLSGAPCQPWASEATYRNVTAEQARNWGLGGHAFCRNPDNDIRPWCFVLNRDRLSWEYCDLAQCQTPTQAAPPTPVSPRLHVPLMPAQPAPPKPQPTTRTPPQSQTPGALPAKREQPPSLTRNGPLSCGQRLRKSLSSMTRVVGGLVALRGAHPYIAALYWGHSFCAGSLIAPCWVLTAAHCLQDRPAPEDLTVVLGQERRNHSCEPCQTLAVRSYRLHEAFSPVSYQHDLALLRLQEDADGSCALLSPYVQPVCLPSGAARPSETTLCQVAGWGHQFEGAEEYASFLQEAQVPFLSLERCSAPDVHGSSILPGMLCAGFLEGGTDACQGDSGGPLVCEDQAAERRLTLQGIISWGSGCGDRNKPGVYTDVAYYLAWIREHTVS

SEQ ID NO: 2 - protein, 597 aa, Mus musculus
MTALLFLGSLLMSLDLTLSAPPWKDSKKFKDAPDGPTVVLTVDGRLCHFPFQYHRQLHHKCIHKRRPGSRPWCATTPNFDEDQQWGYCLEPKKVKDHCSKHNPCHKGGTCINTPNGPHCLCPEHLTGKHCQKEKCFEPQLLKFFHENELWFRTGPGGVARCECKGSEAHCKPVASQACSINPCLNGGSCLLVEDHPLCRCPTGYTGYFCDLDLWATCYEGRGLSYRGQAGTTQSGAPCQRWTVEATYRNMTEKQALSWGLGHHAFCRNPDNDTRPWCFVWSGDRLSWDYCGLEQCQTPTFAPLVVPESQEESPSQAPSLSHAPNDSTDHQTSLSKTNTMGCGQRFRKGLSSFMRVVGGLVALPGSHPYIAALYWGNNFCAGSLIAPCWVLTAAHCLQNRPAPEELTVVLGQDRHNQSCEWCQTLAVRSYRLHEGFSSITYQHDLALLRLQESKTNSCAILSPHVQPVCLPSGAAPPSETVLCEVAGWGHQFEGAEEYSTFLQEAQVPFIALDRCSNSNVHGDAILPGMLCAGFLEGGTDACQGDSGGPLVCEEGTAEHQLTLRGVISWGSGCGDRNKPGVYTDVANYLAWIQKHIAS

SEQ ID NO: 3 - protein, 595 aa, Rattus norvegicus
MTALLFLGSLLMSLDLTLSAPPWKSKEFKDGAGDPSVVLTVDGKLCHFPFQYHRRLYHKCIHKGQPGSRPWCATTPNFDEDQQWGYCLEPKKVKDHCSKHSPCHKGGTCVNTPNGPHCLCPEHLTGKHCQREKCFESQLLKFFHENEIWFRTGPGGVARCQCKGPQAVCKLLTSQVCRVNPCLNGGTCLLVEDHRLCHCPAGYAGPFCDLDLKATCYEDRGLSYRGQAKTTLSGAPCQRWASEATYRNMTETQALSWGLGHHAFCRNPDNDTRPWCYVWSGDRLSWDYCDLEQCQMPTLTSPVSPESHDMLKPRPPILQSSPRDSTRNQNVVSRTSTVVCGQRFRKRLSSLRRVVGGLVALPGSHPYIAALYWGDSFCAGSLIDPCWVLTAAHCLQKRPAPEELTVVLGQDRHNQSCERCQTLAVHSYRLHEGFSSKTYQHDLALLRLRGRKNSCAILSPHVQPVCLPSSAAPPSETVLCEVAGWGHQFEGAEEYATFLQEAQVPFISLDRCSSSNVHGDAILPGMLCAGFLEGGADACQGDSGGPLVCDEGVTERQLTLRGVISWGSGCGDRNKPGVYTDVANYLDWIQEHTAF

SEQ ID NO: 4 - protein, 129 aa, Homo sapiens
EVQLLESGGGLVQPGGSLRLSCAASGFTFSKYIMQWVRQAPGKGLEWVSGIRPSGGTTVYADSVKGRFTISRDNSKNTLYLQMNSLRAEDTAVYYCARALPRSGYLISPHYYYYALDVWGQGTTVTVSS

SEQ ID NO: 5 - protein, 110 aa, Homo sapiens
QSELTQPPSASGTPGQRVTISCSGSSSNIGRNYVYWYQQVPGTAPKLLIYSNNQRPSGVPDRFSGSKSGTSASLVISGLRSEDEADYYCAAWDASLRGVFGGGTKLTVLG

SEQ ID NO: 6 - protein, 5 aa, Homo sapiens
KYIMQ

SEQ ID NO: 7 - protein, 17 aa, Homo sapiens
GIRPSGGTTVYADSVKG

SEQ ID NO: 8 - protein, 17 aa, Artificial
  Heavy chain CDR2 showing variations
  V-segment (3)..(3): Xaa is selected from Arg, Asn, and Asp
  V-segment (4)..(4): Xaa is selcted from Pro, Val, Ile and Met
  V-segment (5)..(5): Xaa is selected from Ser, Pro and Ala
  V-segment (6)..(6): Xaa is selected from Gly, Leu, Val and Thr
  V-segment (7)..(7): Xaa is selected from Gly, Tyr, Gln, Lys, Arg, Asn and Met
  V-segment (8)..(8): Xaa is selected from Thr, Gly and Ser
GIXXXXXXTVYADSVKG

SEQ ID NO: 9 - protein, 20 aa, Homo sapiens
ALPRSGYLISPHYYYYALDV

SEQ ID NO: 10 - protein, 20 aa, Artificial
  Heavy chain CDR3 showing variations
  V-segment (9)..(9): Xaa is selected from Ala, Met and Val
  V-segment (10)..(10): Xaa is selcted from Ser and Lys
  V-segment (11)..(11): Xaa is selected from Pro, Lys, Thr and His
  V-segment (12)..(12): Xaa is selected from His, Asn, Gly and Gln
ALPRSGYLXXXXYYYYALDV

SEQ ID NO: 11 - protein, 13 aa, Homo sapiens
SGSSSNIGRNYVY

SEQ ID NO: 12 - protein, 7 aa, Homo sapiens
SNNQRPS

SEQ ID NO: 13 - protein, 10 aa, Homo sapiens
AAWDASLRGV

SEQ ID NO: 14 - protein, 10 aa, Artificial
  Light chain CDR3 showing variations
  V-segment (2)..(2): Xaa is selected from Ala and Ser
  V-segment (4)..(6): Xaa can be any amino acid
  V-segment (7)..(7): Xaa is selected from Leu and Val
  V-segment (9)..(10): Xaa can be any amino acid
AXWXXXXRXX

SEQ ID NO: 15 - protein, 124 aa, Artificial
  stop template to generate diverse antibodies
  misc_feature (30)..(35): Xaa can be any naturally occurring amino acid (except Cys)
EVQLLESGGGLVQPGGSLRLSCAASGFTFXXXXXXWVRQAPGKGLEWVSGIRPSGGTTVYADSVKGRFTISRDNSKNTLYLQMNSLRAEDTAVYYCARALPRSGYLISPHYYYYALDVWGQGTT

SEQ ID NO: 16 - DNA, 53 bp, Artificial
  Mutagenic trimer mix
  misc_feature (20)..(37): n is a, c, g, or t
agcaagcggttttacctttnnnnnnnnnnnnnnnnnntgggttcgccaggcac

SEQ ID NO: 17 - protein, 133 aa, Artificial
  stop template to generate diverse antibodies
  misc_feature (52)..(57): Xaa can be any naturally occurring amino acid (except Cys)
EVQLLESGGGLVQPGGSLRLSCAASGFTFSKYIMQWVRQAPGKGLEWVSGIXXXXXXTVYADSVKGRFTISRDNSKNTLYLQMNSLRAEDTAVYYCARALPRSGYLISPHYYYYALDVWGQGTTVTVSSASTK

SEQ ID NO: 18 - DNA, 56 bp, Artificial
  Mutagenic trimer mix
  misc_feature (20)..(37): n is a, c, g, or t
ggaatgggttagcggtattnnnnnnnnnnnnnnnnnnaccgtttatgcagatagcg

SEQ ID NO: 19 - protein, 133 aa, Artificial
  stop template to generate diverse antibodies
  misc_feature (100)..(105): Xaa can be any naturally occurring amino acid (except Cys)
EVQLLESGGGLVQPGGSLRLSCAASGFTFSKYIMQWVRQAPGKGLEWVSGIRPSGGTTVYADSVKGRFTISRDNSKNTLYLQMNSLRAEDTAVYYCARAXXXXXXLISPHYYYYALDVWGQGTTVTVSSASTK

SEQ ID NO: 20 - DNA, 57 bp, Artificial
  Mutagenic trimer mix
  misc_feature (20)..(37): n is a, c, g, or t
ttattattgcgcacgtgcannnnnnnnnnnnnnnnnnctgatttctccgcattatta

SEQ ID NO: 21 - protein, 133 aa, Artificial
  stop template to generate diverse antibodies
  misc_feature (105)..(110): Xaa can be any naturally occurring amino acid (except Cys)
EVQLLESGGGLVQPGGSLRLSCAASGFTFSKYIMQWVRQAPGKGLEWVSGIRPSGGTTVYADSVKGRFTISRDNSKNTLYLQMNSLRAEDTAVYYCARALPRSGXXXXXXYYYYALDVWGQGTTVTVSSASTK

SEQ ID NO: 22 - DNA, 56 bp, Artificial
  Mutagenic trimer mix
  misc_feature (18)..(35): n is a, c, g, or t
cactgcctcgtagcggtnnnnnnnnnnnnnnnnnntattattattatgccctggat

SEQ ID NO: 23 - protein, 120 aa, Artificial
  stop template to generate diverse antibodies
  misc_feature (27)..(32): Xaa can be any naturally occurring amino acid (except Cys)
QSVLTQPPSASGTPGQRVTISCSGSSXXXXXXYVYWYQQLPGTAPKLLIYSNNQRPSGVPDRFSGSKSGTSASLAISGLRSEDEADYYCAAWDASLRGVFGGGTKLTVLGQPKAAPSVTL

SEQ ID NO: 24 - DNA, 55 bp, Artificial
  Mutagenic trimer mix
  misc_feature (18)..(35): n is a, c, g, or t
gctgtagcggtagcagcnnnnnnnnnnnnnnnnnntatgtgtattggtatcagca

SEQ ID NO: 25 - protein, 120 aa, Artificial
  stop template to generate diverse antibodies
  misc_feature (90)..(95): Xaa can be any naturally occurring amino acid (except Cys)
QSVLTQPPSASGTPGQRVTISCSGSSSNIGRNYVYWYQQLPGTAPKLLIYSNNQRPSGVPDRFSGSKSGTSASLAISGLRSEDEADYYCXXXXXXLRGVFGGGTKLTVLGQPKAAPSVTL

SEQ ID NO: 26 - DNA, 57 bp, Artificial
  Mutagenic trimer mix
  misc_feature (22)..(39): n is a, c, g, or t
gatgaagccgattattattgtnnnnnnnnnnnnnnnnnnctgcgtggtgtttttggt

SEQ ID NO: 27 - protein, 120 aa, Artificial
  stop template to generate diverse antibodies
  misc_feature (94)..(99): Xaa can be any naturally occurring amino acid (except Cys)
QSVLTQPPSASGTPGQRVTISCSGSSSNIGRNYVYWYQQLPGTAPKLLIYSNNQRPSGVPDRFSGSKSGTSASLAISGLRSEDEADYYCAAWDXXXXXXFGGGTKLTVLGQPKAAPSVTL

SEQ ID NO: 28 - DNA, 55 bp, Artificial
  Mutagenic trimer mix
  misc_feature (20)..(37): n is a, c, g, or t
ttattgtgcagcatgggatnnnnnnnnnnnnnnnnnntttggtggtggcaccaaa

SEQ ID NO: 29 - protein, 17 aa, Artificial
  Affinity-matured HCDR2
GINVPLYGTVYADSVKG

SEQ ID NO: 30 - protein, 17 aa, Artificial
  Affinity-matured HCDR2
GINVPVQGTVYADSVKG

SEQ ID NO: 31 - protein, 17 aa, Artificial
  Affinity-matured HCDR2
GIDIPTKGTVYADSVKG

SEQ ID NO: 32 - protein, 17 aa, Artificial
  Affinity-matured HCDR2
GIDMPTKGTVYADSVKG

SEQ ID NO: 33 - protein, 17 aa, Artificial
  Affinity-matured HCDR2
GINPATRTTVYADSVKG

SEQ ID NO: 34 - protein, 17 aa, Artificial
  Affinity-matured HCDR2
GINPATKTTVYADSVKG

SEQ ID NO: 35 - protein, 17 aa, Artificial
  Affinity-matured HCDR2
GIDVPVRGTVYADSVKG

SEQ ID NO: 36 - protein, 17 aa, Artificial
  Affinity-matured HCDR2
GINPATRSTVYADSVKG

SEQ ID NO: 37 - protein, 17 aa, Artificial
  Affinity-matured HCDR2
GINPATNTTVYADSVKG

SEQ ID NO: 38 - protein, 17 aa, Artificial
  Affinity-matured HCDR2
GINPATMTTVYADSVKG

SEQ ID NO: 39 - protein, 20 aa, Artificial
  Affinity-matured HCDR3
ALPRSGYLMKKNYYYYALDV

SEQ ID NO: 40 - protein, 20 aa, Artificial
  Affinity-matured HCDR3
ALPRSGYLMKTGYYYYALDV

SEQ ID NO: 41 - protein, 20 aa, Artificial
  Affinity-matured HCDR3
ALPRSGYLVKKQYYYYALDV

SEQ ID NO: 42 - protein, 20 aa, Artificial
  Affinity-matured HCDR3
ALPRSGYLVKHGYYYYALDV

SEQ ID NO: 43 - protein, 20 aa, Artificial
  Affinity-matured HCDR3
ALPRSGYLMKPGYYYYALDV

SEQ ID NO: 44 - protein, 13 aa, Artificial
  Affinity-matured LCDR1
SGSSEMTVHHYVY

SEQ ID NO: 45 - protein, 13 aa, Artificial
  Affinity-matured LCDR1
SGSSFSHPHHYVY

SEQ ID NO: 46 - protein, 13 aa, Artificial
  Affinity-matured LCDR1
SGSSEFVEYNYVY

SEQ ID NO: 47 - protein, 13 aa, Artificial
  Affinity-matured LCDR1
SGSSDTNSHHYVY

SEQ ID NO: 48 - protein, 13 aa, Artificial
  Affinity-matured LCDR1
SGSSWTEQHNYVY

SEQ ID NO: 49 - protein, 13 aa, Artificial
  Affinity-matured LCDR1
SGSSVMVTNHYVY

SEQ ID NO: 50 - protein, 13 aa, Artificial
  Affinity-matured LCDR1
SGSSGMVEQNYVY

SEQ ID NO: 51 - protein, 13 aa, Artificial
  Affinity-matured LCDR1
SGSSFKVEETYVY

SEQ ID NO: 52 - protein, 10 aa, Artificial
  Affinity-matured LCDR3
ASWYNDLRGV

SEQ ID NO: 53 - protein, 10 aa, Artificial
  Affinity-matured LCDR3
ASWEIPLRGV

SEQ ID NO: 54 - protein, 10 aa, Artificial
  Affinity-matured LCDR3
ASWTNELRGV

SEQ ID NO: 55 - protein, 10 aa, Artificial
  Affinity-matured LCDR3
ASWWNDLRGV

SEQ ID NO: 56 - protein, 10 aa, Artificial
  Affinity-matured LCDR3
ASWELPLRGV

SEQ ID NO: 57 - protein, 10 aa, Artificial
  Affinity-matured LCDR3
ASWSIPLRGV

SEQ ID NO: 58 - protein, 10 aa, Artificial
  Affinity-matured LCDR3
ASWEVPLRGV

SEQ ID NO: 59 - protein, 10 aa, Artificial
  Affinity-matured LCDR3
AAWDPQVRLA

SEQ ID NO: 60 - protein, 10 aa, Artificial
  Affinity-matured LCDR3
AAWDQQVRLD

SEQ ID NO: 61 - protein, 10 aa, Artificial
  Affinity-matured LCDR3
AAWDQQVRKT

SEQ ID NO: 62 - protein, 10 aa, Artificial
  Affinity-matured LCDR3
AAWDERVRLM

SEQ ID NO: 63 - protein, 10 aa, Artificial
  Affinity-matured LCDR3
AAWDNQVRLG

SEQ ID NO: 64 - DNA, 21 bp, Artificial
  Sequencing primer
gtccttgaccaggcagcccag

SEQ ID NO: 65 - DNA, 21 bp, Artificial
  Sequencing primer
gtgagttagctcactcattag

SEQ ID NO: 66 - DNA, 21 bp, Artificial
  Sequencing primer
ttttcatcggcattttcggtc

SEQ ID NO: 67 - DNA, 24 bp, Artificial
  Sequencing primer
ccatctgatgagcagttgaaatct

SEQ ID NO: 68 - DNA, 24 bp, Artificial
  Sequencing primer
gttcccgccctcctctgaggagct

SEQ ID NO: 69 - DNA, 23 bp, Artificial
  Sequencing primer
agcggataacaatttcacacagg

SEQ ID NO: 70 - DNA, 19 bp, Artificial
  Sequencing primer
ggttctggcaaatattctg

SEQ ID NO: 71 - DNA, 19 bp, Artificial
  Sequencing primer
gttgcaccgaccgaatgta

SEQ ID NO: 72 - DNA, 25 bp, Artificial
  Sequencing primer
accgtgagctggaacagcggtgcgc

SEQ ID NO: 73 - protein, 129 aa, Artificial
  Affinity-matured vH region
EVQLLESGGGLVQPGGSLRLSCAASGFTFSKYIMQWVRQAPGKGLEWVSGIDIPTKGTVYADSVKGRFTISRDNSKNTLYLQMNSLRAEDTAVYYCARALPRSGYLISPHYYYYALDVWGQGTTVTVSS

SEQ ID NO: 74 - protein, 129 aa, Artificial
  Affinity-matured vH region
EVQLLESGGGLVQPGGSLRLSCAASGFTFSKYIMQWVRQAPGKGLEWVSGINVPVQGTVYADSVKGRFTISRDNSKNTLYLQMNSLRAEDTAVYYCARALPRSGYLISPHYYYYALDVWGQGTTVTVSS

SEQ ID NO: 75 - protein, 120 aa, Artificial
  Affinity-matured vL region
QSVLTQPPSASGTPGQRVTISCSGSSEMTVHHYVYWYQQLPGTAPKLLIYSNNQRPSGVPDRFSGSKSGTSASLAISGLRSEDEADYYCAAWDASLRGVFGGGTKLTVLGQPKAAPSVTL

SEQ ID NO: 76 - protein, 130 aa, Artificial
  Affinity-matured vH region
EVQLLESGGGLVQPGGSLRLSCAASGFTFSKYIMQWVRQAPGKGLEWVSGIDMPTKGGTVYADSVKGRFTISRDNSKNTLYLQMNSLRAEDTAVYYCARALPRSGYLISPHYYYYALDVWGQGTTVTVSS

SEQ ID NO: 77 - protein, 131 aa, Artificial
  Affinity-matured vH region
EVQLLESGGGLVQPGGSLRLSCAASGFTFSKYIMQWVRQAPGKGLEWVSGINVPLYGGGTVYADSVKGRFTISRDNSKNTLYLQMNSLRAEDTAVYYCARALPRSGYLISPHYYYYALDVWGQGTTVTVSS